European Patent Application EP 4 799 650 A1, published September 2, 2026. Title: 抗HER2抗体药物偶联物治疗乳腺癌的用途. Applicant: 正大天晴药业集团南京顺欣制药有限公司. The sequence listing filed with the application follows.

SEQUENCE LISTING (21 sequences)

SEQ ID NO: 1 - protein, 10 aa, synthetic construct
  source 1..10: note = HCDR1
GFNIEDTYIH

SEQ ID NO: 2 - protein, 17 aa, synthetic construct
  source 1..17: note = HCDR2
RIYPTNGYTRYADSVKG

SEQ ID NO: 3 - protein, 12 aa, synthetic construct
  source 1..12: note = HCDR3
WGGDGFYAMDYW

SEQ ID NO: 4 - protein, 13 aa, synthetic construct
  source 1..13: note = LCDR1
CRASQDVNTAVAW

SEQ ID NO: 5 - protein, 7 aa, synthetic construct
  source 1..7: note = LCDR2
SASYLYS

SEQ ID NO: 6 - protein, 9 aa, synthetic construct
  source 1..9: note = LCDR3
QQHYTTPPT

SEQ ID NO: 7 - protein, 120 aa, synthetic construct
  source 1..120: note = VH
EVQLVESGGGLVQPGGSLRLSCAASGFNIEDTYIHWVRQAPGKGLEWVARIYPTNGYTRYADSVKGRFTISADTSKNTAYLQMNSLRAEDTAVYYCSRWGGDGFYAMDYWGQGTLVTVSS

SEQ ID NO: 8 - protein, 107 aa, synthetic construct
  source 1..107: note = VL
DIQMTQSPSSLSASVGDRVTITCRASQDVNTAVAWYQQKPGKAPKLLIYSASYLYSGVPSRFSGSRSGTDFTLTISSLQPEDFATYYCQQHYTTPPTFGQGTKVEIK

SEQ ID NO: 9 - protein, 10 aa, synthetic construct
  source 1..10: note = HCDR1
GFTFTDYTMD

SEQ ID NO: 10 - protein, 17 aa, synthetic construct
  source 1..17: note = HCDR2
DVNPNSGGSIYNQRFKG

SEQ ID NO: 11 - protein, 10 aa, synthetic construct
  source 1..10: note = HCDR3
NLGPSFYFDY

SEQ ID NO: 12 - protein, 11 aa, synthetic construct
  source 1..11: note = LCDR1
KASQDVSIGVA

SEQ ID NO: 13 - protein, 7 aa, synthetic construct
  source 1..7: note = LCDR2
SASYRYT

SEQ ID NO: 14 - protein, 9 aa, synthetic construct
  source 1..9: note = LCDR3
QQYYIYPYT

SEQ ID NO: 15 - protein, 119 aa, synthetic construct [sequence omitted]

SEQ ID NO: 16 - protein, 107 aa, synthetic construct [sequence omitted]

SEQ ID NO: 17 - protein, 480 aa, synthetic construct
  source 1..480: note = First polypeptide chain
EVQLVESGGGLVQPGGSLRLSCAASGFNIEDTYIHWVRQAPGKGLEWVARIYPTNGYTRYADSVKGRFTISADTSKNTAYLQMNSLRAEDTAVYYCSRWGGDGFYAMDYWGQGTLVTVSSGGGGSGGGGSGGGGSGGGGSDIQMTQSPSSLSASVGDRVTITCRASQDVNTAVAWYQQKPGKAPKLLIYSASYLYSGVPSRFSGSRSGTDFTLTISSLQPEDFATYYCQQHYTTPPTFGQGTKVEIKGEPKSSDKTHTCPPCPAPELLGGPSVFLFPPKPKDTLMISRTPEVTCVVVDVSHEDPEVKFNWYVDGVEVHNAKTKPREEQYNSTYRVVSVLTVLHQDWLNGKEYKCKVSNKALPAPIEKTISKAKGQPREPQVYTLPPCREEMTKNQVSLWCLVKGFYPSDIAVEWESNGQPENNYKTTPPVLDSDGSFFLYSKLTVDKSRWQQGNVFSCSVMHEALHNHYTQKSLSLSPGK

SEQ ID NO: 18 - protein, 449 aa, synthetic construct
  source 1..449: note = Second polypeptide chain
EVQLVESGGGLVQPGGSLRLSCAASGFTFTDYTMDWVRQAPGKGLEWVADVNPNSGGSIYNQRFKGRFTLSVDRSKNTLYLQMNSLRAEDTAVYYCARNLGPSFYFDYWGQGTLVTVSSASTKGPSVFPLAPSSKSTSGGTAALGCLVKDYFPEPVTVSWNSGALTSGVHTFPAVLQSSGLYSLSSVVTVPSSSLGTQTYICNVNHKPSNTKVDKKVEPKSCDKTHTCPPCPAPELLGGPSVFLFPPKPKDTLMISRTPEVTCVVVDVSHEDPEVKFNWYVDGVEVHNAKTKPREEQYNSTYRVVSVLTVLHQDWLNGKEYKCKVSNKALPAPIEKTISKAKGQPREPQVCTLPPSREEMTKNQVSLSCAVKGFYPSDIAVEWESNGQPENNYKTTPPVLDSDGSFFLVSKLTVDKSRWQQGNVFSCSVMHEALHNRFTQKSLSLSPGK

SEQ ID NO: 19 - protein, 214 aa, synthetic construct
  source 1..214: note = Third polypeptide chain
DIQMTQSPSSLSASVGDRVTITCKASQDVSIGVAWYQQKPGKAPKLLIYSASYRYTGVPSRFSGSGSGTDFTLTISSLQPEDFATYYCQQYYIYPYTFGQGTKVEIKRTVAAPSVFIFPPSDEQLKSGTASVVCLLNNFYPREAKVQWKVDNALQSGNSQESVTEQDSKDSTYSLSSTLTLSKADYEKHKVYACEVTHQGLSSPVTKSFNRGEC

SEQ ID NO: 20 - protein, 479 aa, synthetic construct
  source 1..479: note = First polypeptide chain
EVQLVESGGGLVQPGGSLRLSCAASGFNIEDTYIHWVRQAPGKGLEWVARIYPTNGYTRYADSVKGRFTISADTSKNTAYLQMNSLRAEDTAVYYCSRWGGDGFYAMDYWGQGTLVTVSSGGGGSGGGGSGGGGSGGGGSDIQMTQSPSSLSASVGDRVTITCRASQDVNTAVAWYQQKPGKAPKLLIYSASYLYSGVPSRFSGSRSGTDFTLTISSLQPEDFATYYCQQHYTTPPTFGQGTKVEIKGEPKSSDKTHTCPPCPAPELLGGPSVFLFPPKPKDTLMISRTPEVTCVVVDVSHEDPEVKFNWYVDGVEVHNAKTKPREEQYNSTYRVVSVLTVLHQDWLNGKEYKCKVSNKALPAPIEKTISKAKGQPREPQVYTLPPCREEMTKNQVSLWCLVKGFYPSDIAVEWESNGQPENNYKTTPPVLDSDGSFFLYSKLTVDKSRWQQGNVFSCSVMHEALHNHYTQKSLSLSPG

SEQ ID NO: 21 - protein, 448 aa, synthetic construct
  source 1..448: note = Second polypeptide chain
EVQLVESGGGLVQPGGSLRLSCAASGFTFTDYTMDWVRQAPGKGLEWVADVNPNSGGSIYNQRFKGRFTLSVDRSKNTLYLQMNSLRAEDTAVYYCARNLGPSFYFDYWGQGTLVTVSSASTKGPSVFPLAPSSKSTSGGTAALGCLVKDYFPEPVTVSWNSGALTSGVHTFPAVLQSSGLYSLSSVVTVPSSSLGTQTYICNVNHKPSNTKVDKKVEPKSCDKTHTCPPCPAPELLGGPSVFLFPPKPKDTLMISRTPEVTCVVVDVSHEDPEVKFNWYVDGVEVHNAKTKPREEQYNSTYRVVSVLTVLHQDWLNGKEYKCKVSNKALPAPIEKTISKAKGQPREPQVCTLPPSREEMTKNQVSLSCAVKGFYPSDIAVEWESNGQPENNYKTTPPVLDSDGSFFLVSKLTVDKSRWQQGNVFSCSVMHEALHNRFTQKSLSLSPG